European Patent Application EP 4 803 538 A1, published September 9, 2026. Title: 一种识别人R9AP蛋白的单克隆抗体5E9及其应用. Applicant: 中山大学肿瘤防治中心（中山大学附属肿瘤医院、中山大学肿瘤研究所）. Application CN. The sequence listing filed with the application follows.

SEQUENCE LISTING (26 sequences)

SEQ ID NO: 1 - protein, 210 aa, synthetic construct
MAREECKALLDGLNKTTACYHHLVLTVGGSADSQNLRQELQKTRQKAQELAVSTCARLTAVLRDRGLAADERAEFERLWVAFSGCLDLLEADMRRALELGAAFPLHAPRRPLVRTGVAGASSGVAARALSTRSLRLEAEGDFDVADLRELEREVLQVGEMIDNMEMKVNVPRWTVQARQAAGAELLSTVSAGPSSVVSLQERGGGCDPRK

SEQ ID NO: 2 - DNA, 630 bp, synthetic construct
  source 1..630: mol_type = other DNA
atggcgagggaggagtgcaaggcgctgctggacgggctcaacaagacgactgcgtgctaccaccacctggtgctgaccgtcggtggctcggcggactcgcagaacctgcggcaggagctgcaaaagacgcgccagaaggcgcaggagctggcggtgtccacctgcgcccggctgactgctgtgctgcgcgaccggggcctggccgccgacgagcgcgccgagttcgagcggctctgggtggccttctcgggctgcctggacctgttggaagcggacatgcgacgcgcgctggagctgggcgccgcgttcccgctgcacgcgccgcggcggccgctggtgcgcacaggtgtggctggcgcctcctccggcgtggcggcgcgcgcgctgagcacccgcagcctgcggctcgaggcggagggcgacttcgacgtcgcggacctgcgggagctggagcgcgaggtccttcaggtgggcgagatgatcgacaacatggagatgaaggtcaacgtgccccgctggaccgtgcaagcccggcaggcggcgggcgccgagctcctgtccacggtcagcgccggcccctcctcggtcgtgtccttgcaggagcgcggggggggttgcgaccccaggaag

SEQ ID NO: 3 - protein, 128 aa, synthetic construct
METGLRWLLLVAVLKGVQCQSLEESGGRLVTPGTPLTLSCKASGFDFSSYWMIWVRQAPGEGLEYIGIITKSGNTYYANWAKGRFTISKTSTTVDLKITSPTTEDTATYFCTSNFKLWGQGTLVTVSS

SEQ ID NO: 4 - protein, 109 aa, synthetic construct
QSLEESGGRLVTPGTPLTLSCKASGFDFSSYWMIWVRQAPGEGLEYIGIITKSGNTYYANWAKGRFTISKTSTTVDLKITSPTTEDTATYFCTSNFKLWGQGTLVTVSS

SEQ ID NO: 5 - protein, 5 aa, synthetic construct
SYWMI

SEQ ID NO: 6 - protein, 16 aa, synthetic construct
IITKSGNTYYANWAKG

SEQ ID NO: 7 - protein, 4 aa, synthetic construct
NFKL

SEQ ID NO: 8 - protein, 7 aa, synthetic construct
GFDFSSY

SEQ ID NO: 9 - protein, 5 aa, synthetic construct
TKSGN

SEQ ID NO: 10 - protein, 9 aa, synthetic construct
GGYRYDSDY

SEQ ID NO: 11 - protein, 6 aa, synthetic construct
SSYWMI

SEQ ID NO: 12 - protein, 12 aa, synthetic construct
YIGIITKSGNTY

SEQ ID NO: 13 - protein, 5 aa, synthetic construct
TSNFK

SEQ ID NO: 14 - protein, 132 aa, synthetic construct
MDTRAPTQLLGLLLLWLPGATFAQVLTQTASPVSAAVGGTVTINCQSSQSVYNNNNLAWFQQKPGQPPKVLITSASTLASGVPSRFSGSGSGTQFTLTISDLECDDAAAYYCAGGYSGNIYTFGGGTDVVVK

SEQ ID NO: 15 - protein, 109 aa, synthetic construct
QVLTQTASPVSAAVGGTVTINCQSSQSVYNNNNLAWFQQKPGQPPKVLITSASTLASGVPSRFSGSGSGTQFTLTISDLECDDAAAYYCAGGYSGNIYTFGGGTDVVVK

SEQ ID NO: 16 - protein, 13 aa, synthetic construct
QSSQSVYNNNNLA

SEQ ID NO: 17 - protein, 7 aa, synthetic construct
SASTLAS

SEQ ID NO: 18 - protein, 10 aa, synthetic construct
AGGYSGNIYT

SEQ ID NO: 19 - protein, 9 aa, synthetic construct
YNNNNLAWF

SEQ ID NO: 20 - protein, 10 aa, synthetic construct
VLITSASTLA

SEQ ID NO: 21 - protein, 9 aa, synthetic construct
AGGYSGNIY

SEQ ID NO: 22 - DNA, 70 bp, synthetic construct
  source 1..70: mol_type = other DNA
ggtggttcctctagatcttcctcctctggtggcggtggctcgggcggtggtgggcagtcgbtggaggagt

SEQ ID NO: 23 - DNA, 38 bp, synthetic construct
  source 1..38: mol_type = other DNA
gctggccggcctggccactagttgargagacggtgacc

SEQ ID NO: 24 - DNA, 70 bp, synthetic construct; identical to SEQ ID NO: 22
  source 1..70: mol_type = other DNA

SEQ ID NO: 25 - DNA, 38 bp, synthetic construct; identical to SEQ ID NO: 23
  source 1..38: mol_type = other DNA

SEQ ID NO: 26 - protein, 4 aa, synthetic construct
GGGS